European Patent Application EP 4 393 948 A1, published July 3, 2024. Title: Therapeutic VHH antibodies cross-neutralizing the IL-17A and IL-17F homodimers as well as the IL-17AF heterodimer. Applicant: BiondVax Pharmaceuticals Ltd. Application EP. The sequence listing filed with the application follows.

SEQUENCE LISTING (36 sequences)

SEQ ID NO: 1 - protein, 121 aa, synthetic construct
  REGION 1..121: note = IL-17A homodimer
GSEDSNFPRTVMVNLNIHNRNTNTNPKRSSDYYDRSTSPWNLHRNEDPERYPSVIWEAKCRHLGCINADGNVDYHMNSVPIQQEILVLRREPPHSPNSFRLEKILVSVGCTCVTPIVHHVA

SEQ ID NO: 2 - protein, 130 aa, synthetic construct
  REGION 1..130: note = IL-17F homodimer
GSEGETFFQKPESCPPVPGGSMKLDIGIINENQRVSMSRNIESRSTSPWDYTVTWDPNRYPSEVVQAQCRNLGCINAQGKEDISMNSVPIQQETLVVRRKHQGCSVSFQLEKVLVTVGCTCVTPVIHHVQ

SEQ ID NO: 3 - protein, 121 aa, synthetic construct
  REGION 1..121: note = IL-17A/F heterodimer - two polypeptide units
GSEDSNFPRTVMVNLNIHNRNTNTNPKRSSDYYDRSTSPWNLHRNEDPERYPSVIWEAKCRHLGCINADGNVDYHMNSVPIQQEILVLRREPPHCPNSFRLEKILVSVGCTCVTPIVHHVA

SEQ ID NO: 4 - protein, 130 aa, synthetic construct
  REGION 1..130: note = IL-17F unit
GSEGETFFQKPESCPPVPGGSMKLDIGIINENQRVSMSRNIESRSTSPWDYTVTWDPNRYPSEVVQAQCRNLGCINAQGKEDISMNSVPIQQETLVVRRKHQGSSVSFQLEKVLVTVGCTCVTPVIHHVQ

SEQ ID NO: 5 - protein, 123 aa, synthetic construct
  REGION 1..123: note = VHH antibody sequence, Re42H11
QVQLVESGGGLVQAGGSLRLSCAASGLTASSYAMGWFRQAPGKEREFVAAISWISGGTKYADSVKGRFTMSRDNAKKQVYLEMNSLKPEDTAVYYCNDMPYGLDTRMDEYAYWGQGTQVTVSS

SEQ ID NO: 6 - protein, 15 aa, synthetic construct
  REGION 1..15: note = CDR1_Re42H11
AASGLTASSYAMGWF

SEQ ID NO: 7 - protein, 19 aa, synthetic construct
  REGION 1..19: note = CDR2_Re42H11
FVAAISWISGGTKYADSVK

SEQ ID NO: 8 - protein, 18 aa, synthetic construct
  REGION 1..18: note = CDR3_Re42H11
NDMPYGLDTRMDEYAYWG

SEQ ID NO: 9 - protein, 123 aa, synthetic construct
  REGION 1..123: note = VHH antibody sequence, Bm18A09
QVQLVESGGGLVQAGGSLRLSCAASGLTGSSYAMGWFRQAPGKEREFVAAISWISGSTKYTDSVKDRFTMSRDNAKKQVYLEMNSLKPEDTAVYYCNDMPYGLDTRMDEYVYWGQGTQVTVSS

SEQ ID NO: 10 - protein, 15 aa, synthetic construct
  REGION 1..15: note = CDR1_Bm18A09
AASGLTGSSYAMGWF

SEQ ID NO: 11 - protein, 19 aa, synthetic construct
  REGION 1..19: note = CDR2_Bm18A09
FVAAISWISGSTKYTDSVK

SEQ ID NO: 12 - protein, 18 aa, synthetic construct
  REGION 1..18: note = CDR3_Bm18A09
NDMPYGLDTRMDEYVYWG

SEQ ID NO: 13 - protein, 123 aa, synthetic construct
  REGION 1..123: note = VHH antibody sequence, Re42B03
QVQLVESGGGLVQAGGSLRLSCAASGLTGSSYAMGWFRQAPGKEREFVAAISWISGGTKYTDSVKDRFTMSRDYAKKQVYLEMNSLKPEDTAVYYCNDMPYGLDTRMDEYVYWGQGTQVTVSS

SEQ ID NO: 14 - protein, 15 aa, synthetic construct
  REGION 1..15: note = CDR1_Re42B03
AASGLTGSSYAMGWF

SEQ ID NO: 15 - protein, 19 aa, synthetic construct
  REGION 1..19: note = CDR2_Re42B03
FVAAISWISGGTKYTDSVK

SEQ ID NO: 16 - protein, 18 aa, synthetic construct
  REGION 1..18: note = CDR3_Re42B03
NDMPYGLDTRMDEYVYWG

SEQ ID NO: 17 - protein, 123 aa, synthetic construct
  REGION 1..123: note = VHH antibody sequence, Re42B04
QVQLVESGGGLVQVGGSLRLSCEVSGLPVSSYAMGWFRQAPEKEREFVAAISWIGGDSRYAHFVKGRFTISRDNAKNTVHLQMDSLKPEDTAVYYCNDMPYGLDTRMDEYEYWGLGTQVTVSS

SEQ ID NO: 18 - protein, 15 aa, synthetic construct
  REGION 1..15: note = CDR1_Re42B04
EVSGLPVSSYAMGWF

SEQ ID NO: 19 - protein, 19 aa, synthetic construct
  REGION 1..19: note = CDR2_Re42B04
FVAAISWIGGDSRYAHFVK

SEQ ID NO: 20 - protein, 18 aa, synthetic construct
  REGION 1..18: note = CDR3_Re42B04
NDMPYGLDTRMDEYEYWG

SEQ ID NO: 21 - protein, 123 aa, synthetic construct
  REGION 1..123: note = VHH antibody sequence, Bm18F11
QVQLVESGGDLVQAGGSLRLSCAASGLTGSSYAMGWFRQAPGKEREFVAAISWISGDTKYTDSVKGRFTMSRDNAKKQVYLEMNSLKPEDTAVYYCNDMPYGLDTRMDEYVYWGQGTQVTVSS

SEQ ID NO: 22 - protein, 15 aa, synthetic construct
  REGION 1..15: note = CDR1_Bm18F11
AASGLTGSSYAMGWF

SEQ ID NO: 23 - protein, 19 aa, synthetic construct
  REGION 1..19: note = CDR2_Bm18F11
FVAAISWISGDTKYTDSVK

SEQ ID NO: 24 - protein, 18 aa, synthetic construct
  REGION 1..18: note = CDR3_Bm18F11
NDMPYGLDTRMDEYVYWG

SEQ ID NO: 25 - protein, 123 aa, synthetic construct
  REGION 1..123: note = VHH antibody sequence, Bm18B05
QVQLVESGGGLVQPGGSLRLSCAVSGRTFSSYAMGWFRRPPGKEREFVAAISWSGGDTKYADFVTDRFTISRDDAKSTVYLQMNSLKPEDTAVYYCNDMPYGLDTRMDEYEYWGQGTQVTVSS

SEQ ID NO: 26 - protein, 15 aa, synthetic construct
  REGION 1..15: note = CDR1_Bm18B05
AVSGRTFSSYAMGWF

SEQ ID NO: 27 - protein, 19 aa, synthetic construct
  REGION 1..19: note = CDR2_Bm18B05
FVAAISWSGGDTKYADFVT

SEQ ID NO: 28 - protein, 18 aa, synthetic construct
  REGION 1..18: note = CDR3_Bm18B05
NDMPYGLDTRMDEYEYWG

SEQ ID NO: 29 - protein, 116 aa, synthetic construct
  REGION 1..116: note = VHH antibody sequence, Bm17B02
QVQLVESGGGLVNTGGSLRLSCVVSGHTSEISAMGWYRQAPGKQRELVALITSRSGDTHYSDSVKGRFSISRDNAKNTMYLQMNSLNPDDTAVYYCVHNEPGHLYMAQGTQVTVSS

SEQ ID NO: 30 - protein, 15 aa, synthetic construct
  REGION 1..15: note = CDR1_Bm17B02
VVSGHTSEISAMGWY

SEQ ID NO: 31 - protein, 19 aa, synthetic construct
  REGION 1..19: note = CDR2_Bm17B02
LVALITSRSGDTHYSDSVK

SEQ ID NO: 32 - protein, 11 aa, synthetic construct
  REGION 1..11: note = CDR3_Bm17B02
VHNEPGHLYMA

SEQ ID NO: 33 - protein, 116 aa, synthetic construct
  REGION 1..116: note = VHH antibody sequence, Re42F08
QVQLVESGGGLVKAGGSLRLSCVVSGHTSEISAMGWYRQAPGKQRELVALITSRSGDTHYSDSVKGRFSISRDNAKNTMYLQMNSLNPDDTAVYYCVHNEPGHLYMAQGTQVTVSS

SEQ ID NO: 34 - protein, 15 aa, synthetic construct
  REGION 1..15: note = CDR1_Re42F08
VVSGHTSEISAMGWY

SEQ ID NO: 35 - protein, 19 aa, synthetic construct
  REGION 1..19: note = CDR2_Re42F08
LVALITSRSGDTHYSDSVK

SEQ ID NO: 36 - protein, 11 aa, synthetic construct
  REGION 1..11: note = CDR3_Re42F08
VHNEPGHLYMA